European Patent Application EP 4 249 052 A1, published September 27, 2023. Title: Composition for improving intestinal bacterial flora. Applicant: Teijin Limited. The sequence listing filed with the application follows.

SEQUENCE LISTING (4 sequences)

SEQ ID NO: 1 - DNA, 20 bp, Artificial Sequence
  primer
cacrgtaaacgatggatgcc

SEQ ID NO: 2 - DNA, 16 bp, Artificial Sequence
  primer
ggtcgggttgcagacc

SEQ ID NO: 3 - DNA, 25 bp, Artificial Sequence
  primer
ccgtagatatctggaggaacatcag

SEQ ID NO: 4 - DNA, 25 bp, Artificial Sequence
  primer
acatctagcatccatcgtttacagc